European Patent Application EP 4 617 380 A1, published September 17, 2025. Title: Method for Scanning electron microscopy (SEM)-based optical DNA mapping. Applicant: SOGANG UNIVERSITY RESEARCH FOUNDATION. Application EP. The sequence listing filed with the application follows.

SEQUENCE LISTING (6 sequences)

SEQ ID NO: 1 - protein, 283 aa, synthetic construct
MGSSHHHHHHSSGLVPRGSHMMLPGCMLMVSKGEEDNMASLPATHELHIFGSINGVDFDMVGQGTGNPNDGYEELNLKSTKGDLQFSPWILVPHIGYGFHQYLPYPDGMSPFQAAMVDGSGYQVHRTMQFEDGASLTVNYRYTYEGSHIKGEAQVKGTGFPADGPVMTNSLTAADWCRSKKTYPNDKTIISTFKWSYTTGNGKRYRSTARTTYTFAKPMAANYLKNQPMYVFRKTELKHSKTELNFKEWQKAFTDVMGMDELYKLETPKRPRGRPKKMLGSGC

SEQ ID NO: 2 - protein, 604 aa, synthetic construct
MGSSHHHHHHSSGLVPRGSHMDLRTLGYSQQQQEKIKPKVRSTVAQHHEALVGHGFTHAHIVALSQHPAALGTVAVKYQDMIAALPEATHEAIVGVGKQWSGARALEALLTVAGELRGPPLQLDTGQLLKIAKRGGVTAVEAVHAWRNALTGAPLNLTPAQVVAIASNNGGKQALETVQRLLPVLCQDHGLTPAQVVAIASNGGGKQALETVQRLLPVLCQAHGLTPDQVVAIASHDGGKQALETVQRLLPVLCQDHGLTPAQVVAIASNGGGKQALETVQRLLPVLCQAHGLTPDQVVAIASNNGGKQALETVQRLLPVLCQAHGLTPAQVVAIASNGGGKQALETVQRLLPVLCQDHGGGSGGMVSKGEELFTGVVPILVELDGDVNGHKFSVSGEGEGDATYGKLTLKFICTTGKLPVPWPTLVTTFAYGLQCFARYPDHMKQHDFFKSAMPEGYVQERTISFKDDGNYKTRAEVKFEGDTLVNRIELKGTDFKEDGNILGHKLEYNYNSHNVYITADKQKNGIKANFKIRHNIEDGSVQLADHYQQNTPIGDGPVLLPDNHYLSTQSALSKDPNEKRDHMVLLEFVTAAGITLGMDELYK

SEQ ID NO: 3 - protein, 162 aa, synthetic construct
MGSSHHHHHHSSGLVPRGSHMMSEALKILNNIRTLRAQARECTLETLEEMLEKLEVVVNERREEESAAAAEVEERTRKLQQYREMLIADGIDPNELLNSLAAVKSGTKAKRAQRPAKYSYVDENGETKTWTGQGRTPAVIKKAMDEQGKSLDDFLIKQGSGC

SEQ ID NO: 4 - protein, 396 aa, synthetic construct
MGSSHHHHHHSSGLVPRGSHMMSEALKILNNIRTLRAQARECTLETLEEMLEKLEVVVNERREEESAAAAEVEERTRKLQQYREMLIADGIDPNELLNSLAAVKSGTKAKRAQRPAKYSYVDENGETKTWTGQGRTPAVIKKAMDEQGKSLDDFLIKQEFMVSKGEAVIKEFMRFKVHMEGSMNGHEFEIEGEGEGRPYEGTQTAKLKVTKGGPLPFSWDILSPQFMYGSRAFTKHPADIPDYYKQSFPEGFKWERVMNFEDGGAVTVTQDTSLEDGTLIYKVKLRGTNFPPDGPVMQKKTMGWEASTERLYPEDGVLKGDIKMALRLKDGGRYLADFKTTYKAKKPVQMPGAYNVDRKLDITSHNEDYTVVEQYERSEGRHSTGGMDELYKGSGC

SEQ ID NO: 5 - protein, 334 aa, synthetic construct
MGSSHHHHHHSSGLVPRGSHMMEQRITLKDYAMRFGQTKTAKDLGVYQSAINKAIHAGRKIFLTINADGSVYAEEVKPFPSNKKTTAGGSGGPGMVSKGEEDNMASLPATHELHIFGSINGVDFDMVGQGTGNPNDGYEELNLKSTKGDLQFSPWILVPHIGYGFHQYLPYPDGMSPFQAAMVDGSGYQVHRTMQFEDGASLTVNYRYTYEGSHIKGEAQVKGTGFPADGPVMTNSLTAADWCRSKKTYPNDKTIISTFKWSYTTGNGKRYRSTARTTYTFAKPMAANYLKNQPMYVFRKTELKHSKTELNFKEWQKAFTDVMGMDELYKGSGC

SEQ ID NO: 6 - protein, 5 aa, synthetic construct
GGSGG